European Patent Application EP 4 603 506 A1, published August 20, 2025. Title: Novel GLP-1 receptor antagonist analogs and a pharmaceutical composition for preventing or treating congenital hyperinsulinism (CHI) or hypoglycaemia comprising the same. Applicant: HANMI PHARM. CO., LTD. Application KR. The sequence listing filed with the application follows.

SEQUENCE LISTING (25 sequences)

SEQ ID NO: 1 - protein, 35 aa, synthetic construct
TFTSDLSKQMEEEAVRLFIEWLKNGGPSSGAPPPS

SEQ ID NO: 2 - protein, 33 aa, synthetic construct
TSDLSKQMEEEAVRLFIEWLKNGGPSSGAPPPS

SEQ ID NO: 3 - protein, 31 aa, synthetic construct
DLSKQMEEEAVRLFIEWLKNGGPSSGAPPPS

SEQ ID NO: 4 - protein, 31 aa, synthetic construct
DLSAQMEEEAVRLFIEWLKNGGPSSGAPPPS

SEQ ID NO: 5 - protein, 31 aa, synthetic construct
DLSSQMEEEAVRLFIEWLKNGGPSSGAPPPS

SEQ ID NO: 6 - protein, 27 aa, synthetic construct
QMEEEAVRLFIEWLKNGGPSSGAPPPS

SEQ ID NO: 7 - protein, 33 aa, synthetic construct
TSDVSSYLEEEAVRLFIAWLVKGGPSSGAPPPS

SEQ ID NO: 8 - protein, 31 aa, synthetic construct
DVSSYLEEEAVRLFIAWLVKGGPSSGAPPPS

SEQ ID NO: 9 - protein, 31 aa, synthetic construct
DVSSYLEEQAVREFIAWLVKGGPSSGAPPPS

SEQ ID NO: 10 - protein, 31 aa, synthetic construct
DLSSYLEEEAVRLFIEWLKNGGPSSGAPPPS

SEQ ID NO: 11 - protein, 31 aa, synthetic construct
DVSSYLEEEAVRLFIEWLKNGGPSSGAPPPS

SEQ ID NO: 12 - protein, 32 aa, synthetic construct
DVSSYLEEEAVRLFIAWLVKGGPSSGAPPPSC

SEQ ID NO: 13 - protein, 31 aa, synthetic construct
  SITE 19: note = X is C20diacid-(gamma)Glu-(AEEA)2-Lys
DLSSYLEEEAVRLFIEWLXNGGPSSGAPPPS

SEQ ID NO: 14 - protein, 31 aa, synthetic construct
  SITE 19: note = X is C18diacid-(gamma)Glu-(AEEA)2-Lys
DLSSYLEEEAARLFIEWLXNGGPSSGAPPPS

SEQ ID NO: 15 - protein, 31 aa, synthetic construct
  SITE 20: note = X is C18diacid-(gamma)Glu-(AEEA)2-Lys
DVSSYLEEEAVRLFIAWLVXGGPSSGAPPPS

SEQ ID NO: 16 - protein, 31 aa, synthetic construct
  SITE 20: note = X is C18diacid-(gamma)Glu-(AEEA)2-Lys
DVSSYLEEEAARLFIAWLVXGGPSSGAPPPS

SEQ ID NO: 17 - protein, 32 aa, synthetic construct
  SITE 32: note = X is C18diacid-(gamma)Glu-(AEEA)2-Lys
DLSSYLEEEAVRLFIEWLKNGGPSSGAPPPSX

SEQ ID NO: 18 - protein, 32 aa, synthetic construct
  SITE 32: note = X is C18diacid-(gamma)Glu-(AEEA)2-Lys
DVSSYLEEEAVRLFIAWLVKGGPSSGAPPPSX

SEQ ID NO: 19 - protein, 32 aa, synthetic construct; identical to SEQ ID NO: 17
  SITE 32: note = X is C20diacid-(gamma)Glu-(AEEA)2-Lys

SEQ ID NO: 20 - protein, 32 aa, synthetic construct; identical to SEQ ID NO: 18
  SITE 32: note = X is C20diacid-(gamma)Glu-(AEEA)2-Lys

SEQ ID NO: 21 - protein, 32 aa, synthetic construct; identical to SEQ ID NO: 17
  SITE 32: note = X is C16acid-(gamma)Glu-(AEEA)2-Lys

SEQ ID NO: 22 - protein, 32 aa, synthetic construct; identical to SEQ ID NO: 17
  SITE 32: note = X is C16diacid-(gamma)Glu-(AEEA)2-Lys

SEQ ID NO: 23 - protein, 31 aa, Homo sapiens
HAEGTFTSDVSSYLEGQAAKEFIAWLVKGRG

SEQ ID NO: 24 - protein, 31 aa, synthetic construct; identical to SEQ ID NO: 3

SEQ ID NO: 25 - protein, 36 aa, synthetic construct
  SITE 1: note = X is Thr(T) or absent
  SITE 2: note = X is Phe(F) or absent
  SITE 3: note = X is Thr(T) or absent
  SITE 4: note = X is Ser(S) or absent
  SITE 5: note = X is Asp(D) or absent
  SITE 6: note = X is Leu(L), Val(V), or absent
  SITE 7: note = X is Ser(S) or absent
  SITE 8: note = X is Ala(A), Lys(K), Ser(S), or absent
  SITE 9: note = X is Gln(Q) orTyr(Y)
  SITE 10: note = X is Met(M) or Leu(L)
  SITE 13: note = X is Glu(E) or Gln(Q)
  SITE 15: note = X is Ala(A) or Val(V)
  SITE 17: note = X is Leu(L) or Glu(E)
  SITE 20: note = X is Glu(E) or Ala(A)
  SITE 23: note = X is Lys(K), Val(V), or an acylated amino acid
  SITE 24: note = X is Asn(N), Lys(K), or an anylated amino acid
  SITE 36: note = X is Cys(C), Lys(K), an acylated amino acid or absent
XXXXXXXXXXEEXAXRXFIXWLXXGGPSSGAPPPSX